European Patent Application EP 4 772 535 A1, published July 8, 2026. Title: 靶向受体酪氨酸激酶样孤儿受体1的抗体及其应用. Applicant: 正大天晴药业集团股份有限公司. The sequence listing filed with the application follows.

SEQUENCE LISTING (95 sequences)

SEQ ID NO: 1 - protein, 5 aa, synthetic construct
SYGIT

SEQ ID NO: 2 - protein, 17 aa, synthetic construct
EIYPRSGNTYFNEKFKG

SEQ ID NO: 3 - protein, 10 aa, synthetic construct
DRTGTGVDDY

SEQ ID NO: 4 - protein, 11 aa, synthetic construct
ITNTDIDDDMS

SEQ ID NO: 5 - protein, 7 aa, synthetic construct
EGNTLRP

SEQ ID NO: 6 - protein, 9 aa, synthetic construct
LQSNNLPYT

SEQ ID NO: 7 - protein, 119 aa, synthetic construct
QVQLQQSGTELARPGASVKLSCKASGYTFTSYGITWVKQRTGQGLEWIGEIYPRSGNTYFNEKFKGKATLTADKSSSTAYMELRSLTSEDSAVYFCARDRTGTGVDDYWGQGTTLTVSS

SEQ ID NO: 8 - protein, 107 aa, synthetic construct
DIVLTQSPASLSMAIGEKVTIRCITNTDIDDDMSWYQQKPGEPPNLLISEGNTLRPGVPSRFSSSGYGRDFVFTIENMLSEDVADYYCLQSNNLPYTFGGGTKLEIK

SEQ ID NO: 9 - protein, 5 aa, synthetic construct
NYGIS

SEQ ID NO: 10 - protein, 17 aa, synthetic construct
EIYPRSVNTYYSAKFKG

SEQ ID NO: 11 - protein, 9 aa, synthetic construct
HYYGSSLDY

SEQ ID NO: 12 - protein, 11 aa, synthetic construct
ITSSDIEDDMN

SEQ ID NO: 13 - protein, 7 aa, synthetic construct
EGNSLRP

SEQ ID NO: 14 - protein, 8 aa, synthetic construct
LQSDNIFT

SEQ ID NO: 15 - protein, 118 aa, synthetic construct
EVQLQQSGAELARPGASVKLSCKASGYTFTNYGISWVKQRTGQGLEWIGEIYPRSVNTYYSAKFKGKATLTADKSSSTAYMELRSLTSEDSAVYFCARHYYGSSLDYWGQGTTLTVSS

SEQ ID NO: 16 - protein, 106 aa, synthetic construct
DIVLTQSPASLSVATGEKVTIRCITSSDIEDDMNWYQQKPGEPPKLLISEGNSLRPGVPSRFSSSGYGTDFVFTIENTLSEDVADYYCLQSDNIFTFGSGTKLEIK

SEQ ID NO: 17 - protein, 5 aa, synthetic construct
TYGMA

SEQ ID NO: 18 - protein, 17 aa, synthetic construct
SIHKGGFSTYYPDNVKG

SEQ ID NO: 19 - protein, 9 aa, synthetic construct
HDWDGAMDY

SEQ ID NO: 20 - protein, 11 aa, synthetic construct
KASQDINSYLN

SEQ ID NO: 21 - protein, 7 aa, synthetic construct
RANRLVD

SEQ ID NO: 22 - protein, 9 aa, synthetic construct
LQFDEFPYT

SEQ ID NO: 23 - protein, 118 aa, synthetic construct
DVKLVESGGGLVTPEGSLKLSCAASGFAFSTYGMAWVRQTPEKRLEWVASIHKGGFSTYYPDNVKGRFTISRDNDKNTLYLQMSSLKSEDTAMYYCIRHDWDGAMDYWGQGTSVTVSS

SEQ ID NO: 24 - protein, 107 aa, synthetic construct
DIVLTQSPSSMYASLGERVTITCKASQDINSYLNWFQQKPGKSPKTLIYRANRLVDGVPSRFSGSGSGQDYSLTISSLEYEDLGIYYCLQFDEFPYTFGGGTKLEIK

SEQ ID NO: 25 - protein, 6 aa, synthetic construct
SDYAWN

SEQ ID NO: 26 - protein, 16 aa, synthetic construct
YITYSASTSYNPSLKS

SEQ ID NO: 27 - protein, 9 aa, synthetic construct
GAGTYYFDY

SEQ ID NO: 28 - protein, 11 aa, synthetic construct
ITSTDIDEDMN

SEQ ID NO: 29 - protein, 7 aa, synthetic construct
EDNSLRP

SEQ ID NO: 30 - protein, 9 aa, synthetic construct
LQTNNLPLT

SEQ ID NO: 31 - protein, 118 aa, synthetic construct
DVQLQESGPGLVKPSQSLSLTCTVTGYSITSDYAWNWIRQFPGNKLEWMGYITYSASTSYNPSLKSRISITRDTSKNQFFLQLNSVTTEDTATYYCARGAGTYYFDYWGQGSTLTVSS

SEQ ID NO: 32 - protein, 107 aa, synthetic construct
DIVLTQSPASLSVATGEKVTIRCITSTDIDEDMNWYQQKPGEPPKLLISEDNSLRPGVPSRFSSSGYGTDFVLTIENTLSEDVADYYCLQTNNLPLTFGAGTKLEIK

SEQ ID NO: 33 - protein, 449 aa, synthetic construct
QVQLQQSGTELARPGASVKLSCKASGYTFTSYGITWVKQRTGQGLEWIGEIYPRSGNTYFNEKFKGKATLTADKSSSTAYMELRSLTSEDSAVYFCARDRTGTGVDDYWGQGTTLTVSSASTKGPSVFPLAPSSKSTSGGTAALGCLVKDYFPEPVTVSWNSGALTSGVHTFPAVLQSSGLYSLSSVVTVPSSSLGTQTYICNVNHKPSNTKVDKKVEPKSCDKTHTCPPCPAPELLGGPSVFLFPPKPKDTLMISRTPEVTCVVVDVSHEDPEVKFNWYVDGVEVHNAKTKPREEQYNSTYRVVSVLTVLHQDWLNGKEYKCKVSNKALPAPIEKTISKAKGQPREPQVYTLPPSRDELTKNQVSLTCLVKGFYPSDIAVEWESNGQPENNYKTTPPVLDSDGSFFLYSKLTVDKSRWQQGNVFSCSVMHEALHNHYTQKSLSLSPGK

SEQ ID NO: 34 - DNA, 1347 bp, synthetic construct
  source 1..1347: mol_type = other DNA
caggtgcagctgcagcagtccggcaccgagctggctaggcccggagcttccgtgaagctgagctgcaaggcctccggctataccttcaccagctacggcatcacctgggtgaagcagaggaccggccagggcctggagtggatcggcgagatctatcctaggagcggcaacacctacttcaacgagaagttcaagggcaaggctaccctgaccgccgacaagtcctcctccaccgcctatatggagctgaggtccctgacctccgaggatagcgctgtgtacttctgcgctcgggacaggaccggcaccggcgttgatgactactggggccagggcaccaccctgaccgtgagctccgcctccaccaagggcccctccgtgttccctctggctccttcctccaagtccaccagcggcggcaccgctgccctgggatgtctggtgaaggactacttccctgagcccgtgaccgtgtcttggaatagcggcgctctgacctccggcgtgcacaccttccccgccgtgctgcagtccagcggcctgtatagcctgtccagcgtggtgaccgtgcccagcagctccctgggcacccagacctacatctgtaatgtgaatcacaagcccagcaacaccaaggtggacaagaaggtggagcccaagtcctgtgataagacccacacctgtcccccctgccctgcccctgagctgctgggaggaccttccgtgttcctgttcccccccaagcccaaggacaccctgatgatctcccggacccctgaggtgacctgtgtggtggtggatgtgtcccacgaggaccctgaggtgaagttcaattggtatgtggacggcgtggaggtgcacaatgccaagaccaagcccagggaggagcagtacaacagcacctatcgggtggtgtccgtgctgaccgtgctgcaccaggactggctgaacggcaaggagtacaagtgcaaggtgtccaacaaggccctgcctgctcccatcgagaagaccatcagcaaggccaagggccagcccagggagccccaggtgtataccctgcctcctagccgggacgagctgaccaagaaccaggtgagcctgacctgtctggtgaaaggcttctatcctagcgacatcgccgtggagtgggagtccaatggccagcctgagaataattacaagaccacccctcccgtgctggacagcgacggctccttcttcctgtatagcaagctgaccgtggataagagcaggtggcagcagggcaatgtgttctcctgttccgtgatgcacgaggctctgcacaatcactacacccagaagagcctgagcctgagccccggcaag

SEQ ID NO: 35 - protein, 214 aa, synthetic construct
DIVLTQSPASLSMAIGEKVTIRCITNTDIDDDMSWYQQKPGEPPNLLISEGNTLRPGVPSRFSSSGYGRDFVFTIENMLSEDVADYYCLQSNNLPYTFGGGTKLEIKRTVAAPSVFIFPPSDEQLKSGTASVVCLLNNFYPREAKVQWKVDNALQSGNSQESVTEQDSKDSTYSLSSTLTLSKADYEKHKVYACEVTHQGLSSPVTKSFNRGEC

SEQ ID NO: 36 - DNA, 642 bp, synthetic construct
  source 1..642: mol_type = other DNA
gacatcgtgctgacccagagccctgcctccctgagcatggccatcggcgagaaggtgaccatccggtgtatcaccaacaccgacatcgatgacgacatgagctggtaccagcagaagcctggcgagccccctaacctgctgatctccgagggcaacaccctgaggcccggcgtgccttccaggttcagctccagcggctatggcagggacttcgtgttcaccatcgagaacatgctgagcgaggacgtggccgactattactgcctgcagtccaataacctgccttacaccttcggcggcggcaccaagctggagatcaagcgtacggtggctgcccctagcgtgttcatcttcccccctagcgatgagcagctgaagtccggcaccgccagcgtggtgtgcctgctgaataacttctaccctagggaggccaaggtgcagtggaaggtggataacgccctgcagagcggcaactcccaggagagcgtgaccgagcaggacagcaaggattccacctattccctgtccagcaccctgaccctgagcaaggccgattatgagaagcacaaggtgtacgcctgcgaggtgacccaccagggcctgtccagccctgtgaccaagtccttcaacaggggcgagtgt

SEQ ID NO: 37 - protein, 448 aa, synthetic construct
EVQLQQSGAELARPGASVKLSCKASGYTFTNYGISWVKQRTGQGLEWIGEIYPRSVNTYYSAKFKGKATLTADKSSSTAYMELRSLTSEDSAVYFCARHYYGSSLDYWGQGTTLTVSSASTKGPSVFPLAPSSKSTSGGTAALGCLVKDYFPEPVTVSWNSGALTSGVHTFPAVLQSSGLYSLSSVVTVPSSSLGTQTYICNVNHKPSNTKVDKKVEPKSCDKTHTCPPCPAPELLGGPSVFLFPPKPKDTLMISRTPEVTCVVVDVSHEDPEVKFNWYVDGVEVHNAKTKPREEQYNSTYRVVSVLTVLHQDWLNGKEYKCKVSNKALPAPIEKTISKAKGQPREPQVYTLPPSRDELTKNQVSLTCLVKGFYPSDIAVEWESNGQPENNYKTTPPVLDSDGSFFLYSKLTVDKSRWQQGNVFSCSVMHEALHNHYTQKSLSLSPGK

SEQ ID NO: 38 - DNA, 1344 bp, synthetic construct
  source 1..1344: mol_type = other DNA
gaggtgcagctgcagcagtccggcgctgagctggctcggcctggagctagcgtgaagctgagctgtaaggcttccggctacaccttcaccaactatggcatcagctgggtgaagcagaggaccggccagggcctggagtggatcggcgagatctaccccaggtccgtgaatacctactattccgccaagttcaagggcaaggctaccctgaccgctgacaagagcagctccaccgcctacatggagctgcggtccctgacctccgaggatagcgctgtgtacttctgcgcccggcactactatggcagcagcctggattactggggccagggcaccaccctgaccgtgagctccgcctccaccaagggcccctccgtgttccctctggctccttcctccaagtccaccagcggcggcaccgctgccctgggatgtctggtgaaggactacttccctgagcccgtgaccgtgtcttggaatagcggcgctctgacctccggcgtgcacaccttccccgccgtgctgcagtccagcggcctgtatagcctgtccagcgtggtgaccgtgcccagcagctccctgggcacccagacctacatctgtaatgtgaatcacaagcccagcaacaccaaggtggacaagaaggtggagcccaagtcctgtgataagacccacacctgtcccccctgccctgcccctgagctgctgggaggaccttccgtgttcctgttcccccccaagcccaaggacaccctgatgatctcccggacccctgaggtgacctgtgtggtggtggatgtgtcccacgaggaccctgaggtgaagttcaattggtatgtggacggcgtggaggtgcacaatgccaagaccaagcccagggaggagcagtacaacagcacctatcgggtggtgtccgtgctgaccgtgctgcaccaggactggctgaacggcaaggagtacaagtgcaaggtgtccaacaaggccctgcctgctcccatcgagaagaccatcagcaaggccaagggccagcccagggagccccaggtgtataccctgcctcctagccgggacgagctgaccaagaaccaggtgagcctgacctgtctggtgaaaggcttctatcctagcgacatcgccgtggagtgggagtccaatggccagcctgagaataattacaagaccacccctcccgtgctggacagcgacggctccttcttcctgtatagcaagctgaccgtggataagagcaggtggcagcagggcaatgtgttctcctgttccgtgatgcacgaggctctgcacaatcactacacccagaagagcctgagcctgagccccggcaag

SEQ ID NO: 39 - protein, 213 aa, synthetic construct
DIVLTQSPASLSVATGEKVTIRCITSSDIEDDMNWYQQKPGEPPKLLISEGNSLRPGVPSRFSSSGYGTDFVFTIENTLSEDVADYYCLQSDNIFTFGSGTKLEIKRTVAAPSVFIFPPSDEQLKSGTASVVCLLNNFYPREAKVQWKVDNALQSGNSQESVTEQDSKDSTYSLSSTLTLSKADYEKHKVYACEVTHQGLSSPVTKSFNRGEC

SEQ ID NO: 40 - DNA, 639 bp, synthetic construct
  source 1..639: mol_type = other DNA
gatatcgtgctgacccagtcccccgcctccctgtccgtggctaccggagagaaggtgaccatccggtgtatcacctcctccgatatcgaggacgacatgaactggtatcagcagaagcccggcgagccccctaagctgctgatctccgagggcaatagcctgaggcccggcgtgcctagccggttctcctcctccggctacggcaccgacttcgtgttcaccatcgagaacaccctgagcgaggatgtggccgactactactgtctgcagagcgacaacatcttcaccttcggctccggcaccaagctggagatcaagcgtacggtggctgcccctagcgtgttcatcttcccccctagcgatgagcagctgaagtccggcaccgccagcgtggtgtgcctgctgaataacttctaccctagggaggccaaggtgcagtggaaggtggataacgccctgcagagcggcaactcccaggagagcgtgaccgagcaggacagcaaggattccacctattccctgtccagcaccctgaccctgagcaaggccgattatgagaagcacaaggtgtacgcctgcgaggtgacccaccagggcctgtccagccctgtgaccaagtccttcaacaggggcgagtgt

SEQ ID NO: 41 - protein, 448 aa, synthetic construct
DVKLVESGGGLVTPEGSLKLSCAASGFAFSTYGMAWVRQTPEKRLEWVASIHKGGFSTYYPDNVKGRFTISRDNDKNTLYLQMSSLKSEDTAMYYCIRHDWDGAMDYWGQGTSVTVSSASTKGPSVFPLAPSSKSTSGGTAALGCLVKDYFPEPVTVSWNSGALTSGVHTFPAVLQSSGLYSLSSVVTVPSSSLGTQTYICNVNHKPSNTKVDKKVEPKSCDKTHTCPPCPAPELLGGPSVFLFPPKPKDTLMISRTPEVTCVVVDVSHEDPEVKFNWYVDGVEVHNAKTKPREEQYNSTYRVVSVLTVLHQDWLNGKEYKCKVSNKALPAPIEKTISKAKGQPREPQVYTLPPSRDELTKNQVSLTCLVKGFYPSDIAVEWESNGQPENNYKTTPPVLDSDGSFFLYSKLTVDKSRWQQGNVFSCSVMHEALHNHYTQKSLSLSPGK

SEQ ID NO: 42 - DNA, 1344 bp, synthetic construct
  source 1..1344: mol_type = other DNA
gacgtgaagctggtggagagcggcggcggcctggtgacacctgagggaagcctgaagctgagctgcgccgcctccggcttcgccttctccacctacggcatggcttgggtgcggcagacccctgagaagcggctggagtgggtggccagcatccacaagggcggcttcagcacctactaccccgacaacgtgaagggccggttcaccatctcccgggataatgataagaacaccctgtatctgcagatgtccagcctgaagtccgaggacaccgccatgtactactgcatccggcacgactgggacggcgctatggattattggggccagggcaccagcgtgaccgtgtccagcgcctccaccaagggcccctccgtgttccctctggctccttcctccaagtccaccagcggcggcaccgctgccctgggatgtctggtgaaggactacttccctgagcccgtgaccgtgtcttggaatagcggcgctctgacctccggcgtgcacaccttccccgccgtgctgcagtccagcggcctgtatagcctgtccagcgtggtgaccgtgcccagcagctccctgggcacccagacctacatctgtaatgtgaatcacaagcccagcaacaccaaggtggacaagaaggtggagcccaagtcctgtgataagacccacacctgtcccccctgccctgcccctgagctgctgggaggaccttccgtgttcctgttcccccccaagcccaaggacaccctgatgatctcccggacccctgaggtgacctgtgtggtggtggatgtgtcccacgaggaccctgaggtgaagttcaattggtatgtggacggcgtggaggtgcacaatgccaagaccaagcccagggaggagcagtacaacagcacctatcgggtggtgtccgtgctgaccgtgctgcaccaggactggctgaacggcaaggagtacaagtgcaaggtgtccaacaaggccctgcctgctcccatcgagaagaccatcagcaaggccaagggccagcccagggagccccaggtgtataccctgcctcctagccgggacgagctgaccaagaaccaggtgagcctgacctgtctggtgaaaggcttctatcctagcgacatcgccgtggagtgggagtccaatggccagcctgagaataattacaagaccacccctcccgtgctggacagcgacggctccttcttcctgtatagcaagctgaccgtggataagagcaggtggcagcagggcaatgtgttctcctgttccgtgatgcacgaggctctgcacaatcactacacccagaagagcctgagcctgagccccggcaag

SEQ ID NO: 43 - protein, 214 aa, synthetic construct
DIVLTQSPSSMYASLGERVTITCKASQDINSYLNWFQQKPGKSPKTLIYRANRLVDGVPSRFSGSGSGQDYSLTISSLEYEDLGIYYCLQFDEFPYTFGGGTKLEIKRTVAAPSVFIFPPSDEQLKSGTASVVCLLNNFYPREAKVQWKVDNALQSGNSQESVTEQDSKDSTYSLSSTLTLSKADYEKHKVYACEVTHQGLSSPVTKSFNRGEC

SEQ ID NO: 44 - DNA, 642 bp, synthetic construct
  source 1..642: mol_type = other DNA
gatatcgtgctgacccagagcccttcctccatgtatgctagcctgggcgagagggtgaccatcacctgcaaggctagccaggatatcaatagctacctgaattggttccagcagaagcctggcaagtcccccaagaccctgatctaccgggctaatcggctggtggacggcgtgcccagcaggttctccggctccggatccggccaggactacagcctgaccatctccagcctggagtacgaggacctgggcatctactactgcctgcagttcgatgagttcccctataccttcggcggcggcaccaagctggagatcaagcgtacggtggctgcccctagcgtgttcatcttcccccctagcgatgagcagctgaagtccggcaccgccagcgtggtgtgcctgctgaataacttctaccctagggaggccaaggtgcagtggaaggtggataacgccctgcagagcggcaactcccaggagagcgtgaccgagcaggacagcaaggattccacctattccctgtccagcaccctgaccctgagcaaggccgattatgagaagcacaaggtgtacgcctgcgaggtgacccaccagggcctgtccagccctgtgaccaagtccttcaacaggggcgagtgt

SEQ ID NO: 45 - protein, 448 aa, synthetic construct
DVQLQESGPGLVKPSQSLSLTCTVTGYSITSDYAWNWIRQFPGNKLEWMGYITYSASTSYNPSLKSRISITRDTSKNQFFLQLNSVTTEDTATYYCARGAGTYYFDYWGQGSTLTVSSASTKGPSVFPLAPSSKSTSGGTAALGCLVKDYFPEPVTVSWNSGALTSGVHTFPAVLQSSGLYSLSSVVTVPSSSLGTQTYICNVNHKPSNTKVDKKVEPKSCDKTHTCPPCPAPELLGGPSVFLFPPKPKDTLMISRTPEVTCVVVDVSHEDPEVKFNWYVDGVEVHNAKTKPREEQYNSTYRVVSVLTVLHQDWLNGKEYKCKVSNKALPAPIEKTISKAKGQPREPQVYTLPPSRDELTKNQVSLTCLVKGFYPSDIAVEWESNGQPENNYKTTPPVLDSDGSFFLYSKLTVDKSRWQQGNVFSCSVMHEALHNHYTQKSLSLSPGK

SEQ ID NO: 46 - DNA, 1344 bp, synthetic construct
  source 1..1344: mol_type = other DNA
gatgtgcagctgcaggagtccggccctggcctggtgaagccctcccagagcctgtccctgacctgtaccgtgaccggctactccatcaccagcgattacgcttggaattggatcaggcagttccccggcaacaagctggagtggatgggctacatcacctattccgctagcacctcctataatccctccctgaagagccggatctccatcacccgggacaccagcaagaaccagttcttcctgcagctgaacagcgtgaccaccgaggacaccgccacctattattgtgccaggggcgctggcacctattacttcgattattggggccagggcagcaccctgaccgtgagctccgcctccaccaagggcccctccgtgttccctctggctccttcctccaagtccaccagcggcggcaccgctgccctgggatgtctggtgaaggactacttccctgagcccgtgaccgtgtcttggaatagcggcgctctgacctccggcgtgcacaccttccccgccgtgctgcagtccagcggcctgtatagcctgtccagcgtggtgaccgtgcccagcagctccctgggcacccagacctacatctgtaatgtgaatcacaagcccagcaacaccaaggtggacaagaaggtggagcccaagtcctgtgataagacccacacctgtcccccctgccctgcccctgagctgctgggaggaccttccgtgttcctgttcccccccaagcccaaggacaccctgatgatctcccggacccctgaggtgacctgtgtggtggtggatgtgtcccacgaggaccctgaggtgaagttcaattggtatgtggacggcgtggaggtgcacaatgccaagaccaagcccagggaggagcagtacaacagcacctatcgggtggtgtccgtgctgaccgtgctgcaccaggactggctgaacggcaaggagtacaagtgcaaggtgtccaacaaggccctgcctgctcccatcgagaagaccatcagcaaggccaagggccagcccagggagccccaggtgtataccctgcctcctagccgggacgagctgaccaagaaccaggtgagcctgacctgtctggtgaaaggcttctatcctagcgacatcgccgtggagtgggagtccaatggccagcctgagaataattacaagaccacccctcccgtgctggacagcgacggctccttcttcctgtatagcaagctgaccgtggataagagcaggtggcagcagggcaatgtgttctcctgttccgtgatgcacgaggctctgcacaatcactacacccagaagagcctgagcctgagccccggcaag

SEQ ID NO: 47 - protein, 214 aa, synthetic construct
DIVLTQSPASLSVATGEKVTIRCITSTDIDEDMNWYQQKPGEPPKLLISEDNSLRPGVPSRFSSSGYGTDFVLTIENTLSEDVADYYCLQTNNLPLTFGAGTKLEIKRTVAAPSVFIFPPSDEQLKSGTASVVCLLNNFYPREAKVQWKVDNALQSGNSQESVTEQDSKDSTYSLSSTLTLSKADYEKHKVYACEVTHQGLSSPVTKSFNRGEC

SEQ ID NO: 48 - DNA, 642 bp, synthetic construct
  source 1..642: mol_type = other DNA
gacatcgtgctgacccagtcccccgctagcctgtccgtggctaccggcgagaaggtgaccatccggtgtatcaccagcaccgatatcgacgaggatatgaactggtaccagcagaagcctggcgagcctcctaagctgctgatctccgaggacaactccctgcggcctggcgtgccctccaggttcagctccagcggctacggcaccgacttcgtgctgaccatcgagaacaccctgtccgaggatgtggccgattattactgtctgcagaccaacaatctgcccctgaccttcggcgccggcaccaagctggagatcaagcgtacggtggctgcccctagcgtgttcatcttcccccctagcgatgagcagctgaagtccggcaccgccagcgtggtgtgcctgctgaataacttctaccctagggaggccaaggtgcagtggaaggtggataacgccctgcagagcggcaactcccaggagagcgtgaccgagcaggacagcaaggattccacctattccctgtccagcaccctgaccctgagcaaggccgattatgagaagcacaaggtgtacgcctgcgaggtgacccaccagggcctgtccagccctgtgaccaagtccttcaacaggggcgagtgt

SEQ ID NO: 49 - protein, 17 aa, synthetic construct
EIYPRSVNTYYAQKFQG

SEQ ID NO: 50 - protein, 17 aa, synthetic construct
  VARIANT 12: note = S or A
  VARIANT 13: note = A or Q
  VARIANT 16: note = K or Q
EIYPRSVNTYYXXKFXG

SEQ ID NO: 51 - protein, 118 aa, synthetic construct
QVQLVQSGAEVKKPGSSVKVSCKASGYTFTNYGISWVRQAPGQGLEWMGEIYPRSVNTYYAQKFQGRVTITADKSTSTAYMELSSLRSEDTAVYYCARHYYGSSLDYWGQGTLVTVSS

SEQ ID NO: 52 - protein, 118 aa, synthetic construct
QVQLVQSGAEVKKPGSSVKVSCKASGYTFTNYGISWVRQAPGQGLEWMGEIYPRSVNTYYSAKFKGRVTITADKSTSTAYMELSSLRSEDTAVYYCARHYYGSSLDYWGQGTLVTVSS

SEQ ID NO: 53 - protein, 106 aa, synthetic construct
ETTLTQSPAFMSATPGDKVNISCITSSDIEDDMNWYQQKPGEAAILIISEGNSLRPGIPPRFSSSGYGTDFTLTINNIESEDAAYYFCLQSDNIFTFGQGTKVEIK

SEQ ID NO: 54 - protein, 106 aa, synthetic construct
DIQMTQSPSSLSASVGDRVTITCITSSDIEDDMNWYQQKPGKAPKLLIYEGNSLRPGVPSRFSSSGYGTDFTFTISSLQPEDIATYYCLQSDNIFTFGQGTKVEIK

SEQ ID NO: 55 - protein, 106 aa, synthetic construct
DIQMTQSPSSLSASVGDRVTITCITSSDIEDDMNWYQQKPGKAPKLLISEGNSLRPGVPSRFSSSGYGTDFTFTISSLQPEDIATYYCLQSDNIFTFGQGTKVEIK

SEQ ID NO: 56 - protein, 118 aa, synthetic construct
QVQLVESGGGLVQPGGSLRLSCAASGFAFSTYGMAWVRQAPGKGLEWVASIHKGGFSTYYPDNVKGRFTISRDNAKNSLYLQMNSLRAEDTAVYYCARHDWDGAMDYWGQGTLVTVSS

SEQ ID NO: 57 - protein, 118 aa, synthetic construct
QVQLVESGGGLVQPGGSLRLSCAASGFAFSTYGMAWVRQAPGKGLEWVASIHKGGFSTYYPDNVKGRFTISRDNDKNSLYLQMNSLRAEDTAVYYCIRHDWDGAMDYWGQGTLVTVSS

SEQ ID NO: 58 - protein, 118 aa, synthetic construct
QVQLVESGGGLVQPGGSLRLSCAASGFAFSTYGMAWVRQAPGKRLEWVASIHKGGFSTYYPDNVKGRFTISRDNDKNSLYLQMNSLRAEDTAVYYCIRHDWDGAMDYWGQGTLVTVSS

SEQ ID NO: 59 - protein, 107 aa, synthetic construct
DIQMTQSPSSLSASVGDRVTITCKASQDINSYLNWYQQKPGKAPKTLIYRANRLVDGVPSRFSGSGSGQDYTLTISSLQPEDFATYYCLQFDEFPYTFGQGTKVEIK

SEQ ID NO: 60 - protein, 118 aa, synthetic construct
QVQLQESGPGLVKPSQTLSLTCTVSGYSITSDYAWNWIRQHPGKGLEWIGYITYSASTSYNPSLKSRVTISRDTSKNQFSLKLSSVTAADTAVYYCARGAGTYYFDYWGQGTLVTVSS

SEQ ID NO: 61 - protein, 118 aa, synthetic construct
QVQLQESGPGLVKPSQTLSLTCTVSGYSITSDYAWNWIRQHPGKGLEWIGYITYSASTSYNPSLKSRVTISRDTSKNQFFLKLSSVTAADTAVYYCARGAGTYYFDYWGQGTLVTVSS

SEQ ID NO: 62 - protein, 107 aa, synthetic construct
ETTLTQSPAFMSATPGDKVNISCITSTDIDEDMNWYQQKPGEAAKLIISEDNSLRPGIPPRFSSSGYGTDFTLTINNIESEDAAYYFCLQTNNLPLTFGQGTKVEIK

SEQ ID NO: 63 - protein, 107 aa, synthetic construct
DIQMTQSPSSLSASVGDRVTITCITSTDIDEDMNWYQQKPGKAPKLLIYEDNSLRPGVPSRFSGSGYGTDFTLTISSLQPEDFATYYCLQTNNLPLTFGQGTKVEIK

SEQ ID NO: 64 - protein, 107 aa, synthetic construct
DIQMTQSPSSLSASVGDRVTITCITSTDIDEDMNWYQQKPGKAPKLLISEDNSLRPGVPSRFSSSGYGTDFTLTISSLQPEDFATYYCLQTNNLPLTFGQGTKVEIK

SEQ ID NO: 65 - protein, 448 aa, synthetic construct
QVQLVQSGAEVKKPGSSVKVSCKASGYTFTNYGISWVRQAPGQGLEWMGEIYPRSVNTYYAQKFQGRVTITADKSTSTAYMELSSLRSEDTAVYYCARHYYGSSLDYWGQGTLVTVSSASTKGPSVFPLAPSSKSTSGGTAALGCLVKDYFPEPVTVSWNSGALTSGVHTFPAVLQSSGLYSLSSVVTVPSSSLGTQTYICNVNHKPSNTKVDKKVEPKSCDKTHTCPPCPAPELLGGPSVFLFPPKPKDTLMISRTPEVTCVVVDVSHEDPEVKFNWYVDGVEVHNAKTKPREEQYNSTYRVVSVLTVLHQDWLNGKEYKCKVSNKALPAPIEKTISKAKGQPREPQVYTLPPSRDELTKNQVSLTCLVKGFYPSDIAVEWESNGQPENNYKTTPPVLDSDGSFFLYSKLTVDKSRWQQGNVFSCSVMHEALHNHYTQKSLSLSPGK

SEQ ID NO: 66 - DNA, 1344 bp, synthetic construct
  source 1..1344: mol_type = other DNA
caagtgcaactagtgcaaagtggtgcagaagtcaagaagcccggatcctccgtgaaagtgtcctgcaaggcctctggctacaccttcaccaactacggcatctcctgggtgcggcaggctcctggccagggcctggagtggatgggcgagatctaccctagatctgtgaacacctactacgcccagaagttccagggaagagtgaccatcaccgccgacaagtccacaagcacagcctacatggaactgtcctctctgcggtccgaggataccgctgtgtactactgtgctagacactactatggctctagcctggactactggggccaaggcaccctggtgaccgtgtctagcgcctccaccaagggcccttccgtgttcccactggctccctcttccaagtctacatccggaggaaccgccgctctgggatgcctggtgaaggattatttcccagagcccgtgaccgtgtcttggaactccggcgccctgacaagcggagtgcatacctttcctgctgtgctgcagagctctggcctgtattctctgtccagcgtggtgacagtgccatcttccagcctgggcacccagacatacatctgcaacgtgaatcacaagcctagcaataccaaggtggacaagaaggtggagccaaagtcttgtgataagacccatacatgccccccttgtcctgctccagagctgctgggaggaccatccgtgttcctgtttccacccaagcccaaggacaccctgatgatctcccgcacaccagaggtgacctgcgtggtggtggacgtgagccacgaggatcccgaggtgaagtttaactggtacgtggatggcgtggaggtgcataatgctaagaccaagccaagagaggagcagtataacagcacataccgcgtggtgtctgtgctgaccgtgctgcaccaggactggctgaacggcaaggagtacaagtgcaaggtgtctaataaggccctgcccgctcctatcgagaagacaatctccaaggccaagggccagcctagggagccacaggtgtataccctgcctccatctcgggacgagctgacaaagaaccaggtgtccctgacctgtctggtgaagggcttctaccccagcgatatcgctgtggagtgggagtctaatggccagcctgagaacaattataagaccacaccccctgtgctggacagcgatggctctttctttctgtactctaagctgacagtggataagtccaggtggcagcagggcaacgtgtttagctgctctgtgatgcatgaggctctgcacaatcattacacccagaagtccctgagcctgtctcccggcaag

SEQ ID NO: 67 - protein, 448 aa, synthetic construct
QVQLVQSGAEVKKPGSSVKVSCKASGYTFTNYGISWVRQAPGQGLEWMGEIYPRSVNTYYSAKFKGRVTITADKSTSTAYMELSSLRSEDTAVYYCARHYYGSSLDYWGQGTLVTVSSASTKGPSVFPLAPSSKSTSGGTAALGCLVKDYFPEPVTVSWNSGALTSGVHTFPAVLQSSGLYSLSSVVTVPSSSLGTQTYICNVNHKPSNTKVDKKVEPKSCDKTHTCPPCPAPELLGGPSVFLFPPKPKDTLMISRTPEVTCVVVDVSHEDPEVKFNWYVDGVEVHNAKTKPREEQYNSTYRVVSVLTVLHQDWLNGKEYKCKVSNKALPAPIEKTISKAKGQPREPQVYTLPPSRDELTKNQVSLTCLVKGFYPSDIAVEWESNGQPENNYKTTPPVLDSDGSFFLYSKLTVDKSRWQQGNVFSCSVMHEALHNHYTQKSLSLSPGK

SEQ ID NO: 68 - DNA, 1344 bp, synthetic construct
  source 1..1344: mol_type = other DNA
caagtgcaactagtgcaaagtggtgcagaagtcaagaagcctggctcttctgtgaaagtgtcctgcaaggcctctggctacaccttcaccaactacggcatctcctgggtgcggcaggctcctggacagggcctggagtggatgggcgagatctacccccggtccgtgaacacctactactccgccaagttcaagggcagagtgaccatcaccgctgataagtccacatctacagcctacatggaactgtcctctctgagatccgaggacaccgccgtgtactactgtgctagacactactatggatccagcctggactactggggccagggcaccctggtgaccgtgtctagcgcctccaccaagggcccttccgtgttcccactggctccctcttccaagtctacatccggaggaaccgccgctctgggatgcctggtgaaggattatttcccagagcccgtgaccgtgtcttggaactccggcgccctgacaagcggagtgcatacctttcctgctgtgctgcagagctctggcctgtattctctgtccagcgtggtgacagtgccatcttccagcctgggcacccagacatacatctgcaacgtgaatcacaagcctagcaataccaaggtggacaagaaggtggagccaaagtcttgtgataagacccatacatgccccccttgtcctgctccagagctgctgggaggaccatccgtgttcctgtttccacccaagcccaaggacaccctgatgatctcccgcacaccagaggtgacctgcgtggtggtggacgtgagccacgaggatcccgaggtgaagtttaactggtacgtggatggcgtggaggtgcataatgctaagaccaagccaagagaggagcagtataacagcacataccgcgtggtgtctgtgctgaccgtgctgcaccaggactggctgaacggcaaggagtacaagtgcaaggtgtctaataaggccctgcccgctcctatcgagaagacaatctccaaggccaagggccagcctagggagccacaggtgtataccctgcctccatctcgggacgagctgacaaagaaccaggtgtccctgacctgtctggtgaagggcttctaccccagcgatatcgctgtggagtgggagtctaatggccagcctgagaacaattataagaccacaccccctgtgctggacagcgatggctctttctttctgtactctaagctgacagtggataagtccaggtggcagcagggcaacgtgtttagctgctctgtgatgcatgaggctctgcacaatcattacacccagaagtccctgagcctgtctcccggcaag

SEQ ID NO: 69 - protein, 213 aa, synthetic construct
ETTLTQSPAFMSATPGDKVNISCITSSDIEDDMNWYQQKPGEAAILIISEGNSLRPGIPPRFSSSGYGTDFTLTINNIESEDAAYYFCLQSDNIFTFGQGTKVEIKRTVAAPSVFIFPPSDEQLKSGTASVVCLLNNFYPREAKVQWKVDNALQSGNSQESVTEQDSKDSTYSLSSTLTLSKADYEKHKVYACEVTHQGLSSPVTKSFNRGEC

SEQ ID NO: 70 - DNA, 639 bp, synthetic construct
  source 1..639: mol_type = other DNA
gaaactactctaactcaaagtccagcatttatgtctgctacccctggcgacaaagtgaatatcagctgtatcacctcttctgacatcgaggacgacatgaactggtaccagcagaagcccggcgaggccgccatcctgatcatctccgaaggcaactccctgcggccaggaatccctcctagattctccagctctggctacggcaccgattttacactgaccatcaacaacattgagtccgaggatgctgcctactacttctgcctgcagtccgacaacatcttcaccttcggccaaggcaccaaggtggaaatcaagcgtacggtggccgctcccagcgtgttcatctttcccccttctgacgagcagctgaagtctggcaccgcttccgtggtgtgcctgctgaacaatttctaccccagagaggccaaggtgcagtggaaggtggataacgctctgcagtccggcaatagccaggagtctgtgaccgagcaggactccaaggatagcacatattctctgtcttccaccctgacactgtctaaggccgactacgagaagcacaaggtgtatgcttgcgaggtgacccatcagggcctgagctctcctgtgacaaagtcctttaatcgcggcgagtgt

SEQ ID NO: 71 - protein, 213 aa, synthetic construct
DIQMTQSPSSLSASVGDRVTITCITSSDIEDDMNWYQQKPGKAPKLLIYEGNSLRPGVPSRFSSSGYGTDFTFTISSLQPEDIATYYCLQSDNIFTFGQGTKVEIKRTVAAPSVFIFPPSDEQLKSGTASVVCLLNNFYPREAKVQWKVDNALQSGNSQESVTEQDSKDSTYSLSSTLTLSKADYEKHKVYACEVTHQGLSSPVTKSFNRGEC

SEQ ID NO: 72 - DNA, 639 bp, synthetic construct
  source 1..639: mol_type = other DNA
gatatccaaatgactcaaagtccaagtagtctgtccgcttctgtcggagatagagtgaccatcacctgtatcacctcctccgacatcgaggacgacatgaactggtatcagcagaagcccggcaaggcccctaagctgctgatctacgagggcaactccctgagacctggcgtgccatctcggttctccagctctggctacggcaccgacttcacctttacaatctcctctctgcagcctgaggatatcgccacctactactgcctgcaaagcgacaacatcttcaccttcggccagggcacaaaagtggaaatcaagcgtacggtggccgctcccagcgtgttcatctttcccccttctgacgagcagctgaagtctggcaccgcttccgtggtgtgcctgctgaacaatttctaccccagagaggccaaggtgcagtggaaggtggataacgctctgcagtccggcaatagccaggagtctgtgaccgagcaggactccaaggatagcacatattctctgtcttccaccctgacactgtctaaggccgactacgagaagcacaaggtgtatgcttgcgaggtgacccatcagggcctgagctctcctgtgacaaagtcctttaatcgcggcgagtgt

SEQ ID NO: 73 - protein, 213 aa, synthetic construct
DIQMTQSPSSLSASVGDRVTITCITSSDIEDDMNWYQQKPGKAPKLLISEGNSLRPGVPSRFSSSGYGTDFTFTISSLQPEDIATYYCLQSDNIFTFGQGTKVEIKRTVAAPSVFIFPPSDEQLKSGTASVVCLLNNFYPREAKVQWKVDNALQSGNSQESVTEQDSKDSTYSLSSTLTLSKADYEKHKVYACEVTHQGLSSPVTKSFNRGEC

SEQ ID NO: 74 - DNA, 639 bp, synthetic construct
  source 1..639: mol_type = other DNA
gatatccaaatgactcaaagtccaagtagtctgtctgcttctgtgggcgacagagtgaccatcacctgtatcacctccagcgatatcgaggacgacatgaactggtaccagcagaaacctggcaaggcccctaagctgctgatctccgagggcaactccctgagaccaggagtcccctctcggttctcctcctctggctacggcaccgacttcacatttacaatcagctctctgcagcctgaggatatcgccacctactactgcctgcaatccgacaacatcttcaccttcggccagggcaccaaggtggaaatcaagcgtacggtggccgctcccagcgtgttcatctttcccccttctgacgagcagctgaagtctggcaccgcttccgtggtgtgcctgctgaacaatttctaccccagagaggccaaggtgcagtggaaggtggataacgctctgcagtccggcaatagccaggagtctgtgaccgagcaggactccaaggatagcacatattctctgtcttccaccctgacactgtctaaggccgactacgagaagcacaaggtgtatgcttgcgaggtgacccatcagggcctgagctctcctgtgacaaagtcctttaatcgcggcgagtgt

SEQ ID NO: 75 - protein, 448 aa, synthetic construct
QVQLVESGGGLVQPGGSLRLSCAASGFAFSTYGMAWVRQAPGKGLEWVASIHKGGFSTYYPDNVKGRFTISRDNAKNSLYLQMNSLRAEDTAVYYCARHDWDGAMDYWGQGTLVTVSSASTKGPSVFPLAPSSKSTSGGTAALGCLVKDYFPEPVTVSWNSGALTSGVHTFPAVLQSSGLYSLSSVVTVPSSSLGTQTYICNVNHKPSNTKVDKKVEPKSCDKTHTCPPCPAPELLGGPSVFLFPPKPKDTLMISRTPEVTCVVVDVSHEDPEVKFNWYVDGVEVHNAKTKPREEQYNSTYRVVSVLTVLHQDWLNGKEYKCKVSNKALPAPIEKTISKAKGQPREPQVYTLPPSRDELTKNQVSLTCLVKGFYPSDIAVEWESNGQPENNYKTTPPVLDSDGSFFLYSKLTVDKSRWQQGNVFSCSVMHEALHNHYTQKSLSLSPGK

SEQ ID NO: 76 - DNA, 1344 bp, synthetic construct
  source 1..1344: mol_type = other DNA
caagtgcaactagtggaaagtggtggtggtctcgtgcagcctggaggatctctgcggctgtcttgtgctgcttctggcttcgccttttctacctacggcatggcctgggtccgccaagctcctggcaagggcctggaatgggtggcctccatccacaagggcggcttctccacctattaccccgataatgtgaaaggcagattcaccatctcccgggacaacgccaagaactccctgtacctgcagatgaacagcctgagagccgaggacaccgccgtgtactactgcgccagacacgattgggacggcgctatggactactggggccagggcaccctggtgacagtgtccagcgcctccaccaagggcccttccgtgttcccactggctccctcttccaagtctacatccggaggaaccgccgctctgggatgcctggtgaaggattatttcccagagcccgtgaccgtgtcttggaactccggcgccctgacaagcggagtgcatacctttcctgctgtgctgcagagctctggcctgtattctctgtccagcgtggtgacagtgccatcttccagcctgggcacccagacatacatctgcaacgtgaatcacaagcctagcaataccaaggtggacaagaaggtggagccaaagtcttgtgataagacccatacatgccccccttgtcctgctccagagctgctgggaggaccatccgtgttcctgtttccacccaagcccaaggacaccctgatgatctcccgcacaccagaggtgacctgcgtggtggtggacgtgagccacgaggatcccgaggtgaagtttaactggtacgtggatggcgtggaggtgcataatgctaagaccaagccaagagaggagcagtataacagcacataccgcgtggtgtctgtgctgaccgtgctgcaccaggactggctgaacggcaaggagtacaagtgcaaggtgtctaataaggccctgcccgctcctatcgagaagacaatctccaaggccaagggccagcctagggagccacaggtgtataccctgcctccatctcgggacgagctgacaaagaaccaggtgtccctgacctgtctggtgaagggcttctaccccagcgatatcgctgtggagtgggagtctaatggccagcctgagaacaattataagaccacaccccctgtgctggacagcgatggctctttctttctgtactctaagctgacagtggataagtccaggtggcagcagggcaacgtgtttagctgctctgtgatgcatgaggctctgcacaatcattacacccagaagtccctgagcctgtctcccggcaag

SEQ ID NO: 77 - protein, 448 aa, synthetic construct
QVQLVESGGGLVQPGGSLRLSCAASGFAFSTYGMAWVRQAPGKGLEWVASIHKGGFSTYYPDNVKGRFTISRDNDKNSLYLQMNSLRAEDTAVYYCIRHDWDGAMDYWGQGTLVTVSSASTKGPSVFPLAPSSKSTSGGTAALGCLVKDYFPEPVTVSWNSGALTSGVHTFPAVLQSSGLYSLSSVVTVPSSSLGTQTYICNVNHKPSNTKVDKKVEPKSCDKTHTCPPCPAPELLGGPSVFLFPPKPKDTLMISRTPEVTCVVVDVSHEDPEVKFNWYVDGVEVHNAKTKPREEQYNSTYRVVSVLTVLHQDWLNGKEYKCKVSNKALPAPIEKTISKAKGQPREPQVYTLPPSRDELTKNQVSLTCLVKGFYPSDIAVEWESNGQPENNYKTTPPVLDSDGSFFLYSKLTVDKSRWQQGNVFSCSVMHEALHNHYTQKSLSLSPGK

SEQ ID NO: 78 - DNA, 1344 bp, synthetic construct
  source 1..1344: mol_type = other DNA
caagtgcaactagtggaaagtggtggtggtctcgtgcagcctggaggaagcctgcggctgtcttgtgctgcttctggcttcgccttttctacatatggcatggcctgggtccgccaagctcctggcaagggcctggaatgggtggcctccatccacaagggcggcttctccacctactaccccgataatgtgaaaggcagattcaccatctcccgggacaacgacaagaactccctgtacctgcagatgaactctctgagagccgaggacaccgccgtgtactactgcatcagacacgattgggacggcgctatggactactggggccagggcaccctggtgaccgtgtccagcgcctccaccaagggcccttccgtgttcccactggctccctcttccaagtctacatccggaggaaccgccgctctgggatgcctggtgaaggattatttcccagagcccgtgaccgtgtcttggaactccggcgccctgacaagcggagtgcatacctttcctgctgtgctgcagagctctggcctgtattctctgtccagcgtggtgacagtgccatcttccagcctgggcacccagacatacatctgcaacgtgaatcacaagcctagcaataccaaggtggacaagaaggtggagccaaagtcttgtgataagacccatacatgccccccttgtcctgctccagagctgctgggaggaccatccgtgttcctgtttccacccaagcccaaggacaccctgatgatctcccgcacaccagaggtgacctgcgtggtggtggacgtgagccacgaggatcccgaggtgaagtttaactggtacgtggatggcgtggaggtgcataatgctaagaccaagccaagagaggagcagtataacagcacataccgcgtggtgtctgtgctgaccgtgctgcaccaggactggctgaacggcaaggagtacaagtgcaaggtgtctaataaggccctgcccgctcctatcgagaagacaatctccaaggccaagggccagcctagggagccacaggtgtataccctgcctccatctcgggacgagctgacaaagaaccaggtgtccctgacctgtctggtgaagggcttctaccccagcgatatcgctgtggagtgggagtctaatggccagcctgagaacaattataagaccacaccccctgtgctggacagcgatggctctttctttctgtactctaagctgacagtggataagtccaggtggcagcagggcaacgtgtttagctgctctgtgatgcatgaggctctgcacaatcattacacccagaagtccctgagcctgtctcccggcaag

SEQ ID NO: 79 - protein, 448 aa, synthetic construct
QVQLVESGGGLVQPGGSLRLSCAASGFAFSTYGMAWVRQAPGKRLEWVASIHKGGFSTYYPDNVKGRFTISRDNDKNSLYLQMNSLRAEDTAVYYCIRHDWDGAMDYWGQGTLVTVSSASTKGPSVFPLAPSSKSTSGGTAALGCLVKDYFPEPVTVSWNSGALTSGVHTFPAVLQSSGLYSLSSVVTVPSSSLGTQTYICNVNHKPSNTKVDKKVEPKSCDKTHTCPPCPAPELLGGPSVFLFPPKPKDTLMISRTPEVTCVVVDVSHEDPEVKFNWYVDGVEVHNAKTKPREEQYNSTYRVVSVLTVLHQDWLNGKEYKCKVSNKALPAPIEKTISKAKGQPREPQVYTLPPSRDELTKNQVSLTCLVKGFYPSDIAVEWESNGQPENNYKTTPPVLDSDGSFFLYSKLTVDKSRWQQGNVFSCSVMHEALHNHYTQKSLSLSPGK

SEQ ID NO: 80 - DNA, 1344 bp, synthetic construct
  source 1..1344: mol_type = other DNA
caagtgcaactagtggaaagtggtggtggtctcgtgcagcctggcggctctctgagactgtcttgtgctgcttctggcttcgccttctccacatacggcatggcctgggtcagacaagctcccggcaagcggctggaatgggtggcctccatccacaaaggaggattttctacctactatcctgacaacgtgaagggcagattcaccatctccagagataatgacaagaactccctgtacctgcagatgaacagcctgcgggccgaggacaccgccgtgtactactgcatccggcacgattgggacggcgctatggactactggggccagggcaccctggtgaccgtgtccagcgcctccaccaagggcccttccgtgttcccactggctccctcttccaagtctacatccggaggaaccgccgctctgggatgcctggtgaaggattatttcccagagcccgtgaccgtgtcttggaactccggcgccctgacaagcggagtgcatacctttcctgctgtgctgcagagctctggcctgtattctctgtccagcgtggtgacagtgccatcttccagcctgggcacccagacatacatctgcaacgtgaatcacaagcctagcaataccaaggtggacaagaaggtggagccaaagtcttgtgataagacccatacatgccccccttgtcctgctccagagctgctgggaggaccatccgtgttcctgtttccacccaagcccaaggacaccctgatgatctcccgcacaccagaggtgacctgcgtggtggtggacgtgagccacgaggatcccgaggtgaagtttaactggtacgtggatggcgtggaggtgcataatgctaagaccaagccaagagaggagcagtataacagcacataccgcgtggtgtctgtgctgaccgtgctgcaccaggactggctgaacggcaaggagtacaagtgcaaggtgtctaataaggccctgcccgctcctatcgagaagacaatctccaaggccaagggccagcctagggagccacaggtgtataccctgcctccatctcgggacgagctgacaaagaaccaggtgtccctgacctgtctggtgaagggcttctaccccagcgatatcgctgtggagtgggagtctaatggccagcctgagaacaattataagaccacaccccctgtgctggacagcgatggctctttctttctgtactctaagctgacagtggataagtccaggtggcagcagggcaacgtgtttagctgctctgtgatgcatgaggctctgcacaatcattacacccagaagtccctgagcctgtctcccggcaag

SEQ ID NO: 81 - protein, 214 aa, synthetic construct
DIQMTQSPSSLSASVGDRVTITCKASQDINSYLNWYQQKPGKAPKTLIYRANRLVDGVPSRFSGSGSGQDYTLTISSLQPEDFATYYCLQFDEFPYTFGQGTKVEIKRTVAAPSVFIFPPSDEQLKSGTASVVCLLNNFYPREAKVQWKVDNALQSGNSQESVTEQDSKDSTYSLSSTLTLSKADYEKHKVYACEVTHQGLSSPVTKSFNRGEC

SEQ ID NO: 82 - DNA, 642 bp, synthetic construct
  source 1..642: mol_type = other DNA
gatatccaaatgactcaaagtccaagtagtctgtccgcctccgtgggcgacagagtcacaatcacctgtaaggcctcccaggatatcaactcctacctgaactggtaccagcagaagcctggcaaggctcctaagaccctgatctacagagccaaccggctggtggacggcgtgccatctcggttctccggctctggatctggccaagattatacactgaccatctccagcctccagcctgaggacttcgccacctactactgcctgcagttcgacgagtttccctacaccttcggccagggcaccaaggtggaaatcaagcgtacggtggccgctcccagcgtgttcatctttcccccttctgacgagcagctgaagtctggcaccgcttccgtggtgtgcctgctgaacaatttctaccccagagaggccaaggtgcagtggaaggtggataacgctctgcagtccggcaatagccaggagtctgtgaccgagcaggactccaaggatagcacatattctctgtcttccaccctgacactgtctaaggccgactacgagaagcacaaggtgtatgcttgcgaggtgacccatcagggcctgagctctcctgtgacaaagtcctttaatcgcggcgagtgt

SEQ ID NO: 83 - protein, 448 aa, synthetic construct
QVQLQESGPGLVKPSQTLSLTCTVSGYSITSDYAWNWIRQHPGKGLEWIGYITYSASTSYNPSLKSRVTISRDTSKNQFSLKLSSVTAADTAVYYCARGAGTYYFDYWGQGTLVTVSSASTKGPSVFPLAPSSKSTSGGTAALGCLVKDYFPEPVTVSWNSGALTSGVHTFPAVLQSSGLYSLSSVVTVPSSSLGTQTYICNVNHKPSNTKVDKKVEPKSCDKTHTCPPCPAPELLGGPSVFLFPPKPKDTLMISRTPEVTCVVVDVSHEDPEVKFNWYVDGVEVHNAKTKPREEQYNSTYRVVSVLTVLHQDWLNGKEYKCKVSNKALPAPIEKTISKAKGQPREPQVYTLPPSRDELTKNQVSLTCLVKGFYPSDIAVEWESNGQPENNYKTTPPVLDSDGSFFLYSKLTVDKSRWQQGNVFSCSVMHEALHNHYTQKSLSLSPGK

SEQ ID NO: 84 - DNA, 1344 bp, synthetic construct
  source 1..1344: mol_type = other DNA
caagtgcaactacaagaaagtggtccaggtctggtgaagccttctcagaccctgtctctgacctgtaccgtgtctggctactccatcacctctgactacgcctggaactggatccggcaacaccctggcaaaggactcgagtggatcggctacatcacatattctgcctctaccagctacaaccccagcctgaagtccagagtgaccatctcccgggacacctccaagaaccagttctccctgaagctgtcctccgtgaccgctgctgataccgccgtgtactactgcgccagaggcgctggcacctactacttcgactactggggccagggcacactggtcacagtgtccagcgcctccaccaagggcccttccgtgttcccactggctccctcttccaagtctacatccggaggaaccgccgctctgggatgcctggtgaaggattatttcccagagcccgtgaccgtgtcttggaactccggcgccctgacaagcggagtgcatacctttcctgctgtgctgcagagctctggcctgtattctctgtccagcgtggtgacagtgccatcttccagcctgggcacccagacatacatctgcaacgtgaatcacaagcctagcaataccaaggtggacaagaaggtggagccaaagtcttgtgataagacccatacatgccccccttgtcctgctccagagctgctgggaggaccatccgtgttcctgtttccacccaagcccaaggacaccctgatgatctcccgcacaccagaggtgacctgcgtggtggtggacgtgagccacgaggatcccgaggtgaagtttaactggtacgtggatggcgtggaggtgcataatgctaagaccaagccaagagaggagcagtataacagcacataccgcgtggtgtctgtgctgaccgtgctgcaccaggactggctgaacggcaaggagtacaagtgcaaggtgtctaataaggccctgcccgctcctatcgagaagacaatctccaaggccaagggccagcctagggagccacaggtgtataccctgcctccatctcgggacgagctgacaaagaaccaggtgtccctgacctgtctggtgaagggcttctaccccagcgatatcgctgtggagtgggagtctaatggccagcctgagaacaattataagaccacaccccctgtgctggacagcgatggctctttctttctgtactctaagctgacagtggataagtccaggtggcagcagggcaacgtgtttagctgctctgtgatgcatgaggctctgcacaatcattacacccagaagtccctgagcctgtctcccggcaag

SEQ ID NO: 85 - protein, 448 aa, synthetic construct
QVQLQESGPGLVKPSQTLSLTCTVSGYSITSDYAWNWIRQHPGKGLEWIGYITYSASTSYNPSLKSRVTISRDTSKNQFFLKLSSVTAADTAVYYCARGAGTYYFDYWGQGTLVTVSSASTKGPSVFPLAPSSKSTSGGTAALGCLVKDYFPEPVTVSWNSGALTSGVHTFPAVLQSSGLYSLSSVVTVPSSSLGTQTYICNVNHKPSNTKVDKKVEPKSCDKTHTCPPCPAPELLGGPSVFLFPPKPKDTLMISRTPEVTCVVVDVSHEDPEVKFNWYVDGVEVHNAKTKPREEQYNSTYRVVSVLTVLHQDWLNGKEYKCKVSNKALPAPIEKTISKAKGQPREPQVYTLPPSRDELTKNQVSLTCLVKGFYPSDIAVEWESNGQPENNYKTTPPVLDSDGSFFLYSKLTVDKSRWQQGNVFSCSVMHEALHNHYTQKSLSLSPGK

SEQ ID NO: 86 - DNA, 1344 bp, synthetic construct
  source 1..1344: mol_type = other DNA
caagtgcaactacaagaaagtggtccaggtctcgtgaagccttctcagaccctgtctctgacctgtacagtgtctggatactccatcacctctgactacgcctggaactggatccggcaacaccctggcaagggcctggagtggatcggctacatcacctattctgcctctacctcctacaaccccagcctgaaatccagagtgaccatctcccgggacacctccaagaaccagttctttctgaagctgtcctccgtgacagctgctgataccgccgtgtactactgcgccagaggcgctggcacctactacttcgactactggggccagggcacactggtcaccgtgtccagcgcctccaccaagggcccttccgtgttcccactggctccctcttccaagtctacatccggaggaaccgccgctctgggatgcctggtgaaggattatttcccagagcccgtgaccgtgtcttggaactccggcgccctgacaagcggagtgcatacctttcctgctgtgctgcagagctctggcctgtattctctgtccagcgtggtgacagtgccatcttccagcctgggcacccagacatacatctgcaacgtgaatcacaagcctagcaataccaaggtggacaagaaggtggagccaaagtcttgtgataagacccatacatgccccccttgtcctgctccagagctgctgggaggaccatccgtgttcctgtttccacccaagcccaaggacaccctgatgatctcccgcacaccagaggtgacctgcgtggtggtggacgtgagccacgaggatcccgaggtgaagtttaactggtacgtggatggcgtggaggtgcataatgctaagaccaagccaagagaggagcagtataacagcacataccgcgtggtgtctgtgctgaccgtgctgcaccaggactggctgaacggcaaggagtacaagtgcaaggtgtctaataaggccctgcccgctcctatcgagaagacaatctccaaggccaagggccagcctagggagccacaggtgtataccctgcctccatctcgggacgagctgacaaagaaccaggtgtccctgacctgtctggtgaagggcttctaccccagcgatatcgctgtggagtgggagtctaatggccagcctgagaacaattataagaccacaccccctgtgctggacagcgatggctctttctttctgtactctaagctgacagtggataagtccaggtggcagcagggcaacgtgtttagctgctctgtgatgcatgaggctctgcacaatcattacacccagaagtccctgagcctgtctcccggcaag

SEQ ID NO: 87 - protein, 214 aa, synthetic construct
ETTLTQSPAFMSATPGDKVNISCITSTDIDEDMNWYQQKPGEAAKLIISEDNSLRPGIPPRFSSSGYGTDFTLTINNIESEDAAYYFCLQTNNLPLTFGQGTKVEIKRTVAAPSVFIFPPSDEQLKSGTASVVCLLNNFYPREAKVQWKVDNALQSGNSQESVTEQDSKDSTYSLSSTLTLSKADYEKHKVYACEVTHQGLSSPVTKSFNRGEC

SEQ ID NO: 88 - DNA, 642 bp, synthetic construct
  source 1..642: mol_type = other DNA
gaaactactctaactcaaagtccagcatttatgtccgctacccctggcgacaaggtgaacatttcttgtatcacctctacagatatcgacgaggacatgaactggtaccagcagaagcccggcgaggccgccaagctgatcatctccgaggacaactccctgagaccaggcatccctcctcggtttagcagctctggctacggcaccgacttcaccctgaccatcaacaatatcgagtccgaagatgctgcctactacttctgcctgcagaccaacaacctgcctctgaccttcggccaaggaacaaaagtggaaatcaagcgtacggtggccgctcccagcgtgttcatctttcccccttctgacgagcagctgaagtctggcaccgcttccgtggtgtgcctgctgaacaatttctaccccagagaggccaaggtgcagtggaaggtggataacgctctgcagtccggcaatagccaggagtctgtgaccgagcaggactccaaggatagcacatattctctgtcttccaccctgacactgtctaaggccgactacgagaagcacaaggtgtatgcttgcgaggtgacccatcagggcctgagctctcctgtgacaaagtcctttaatcgcggcgagtgt

SEQ ID NO: 89 - protein, 214 aa, synthetic construct
DIQMTQSPSSLSASVGDRVTITCITSTDIDEDMNWYQQKPGKAPKLLIYEDNSLRPGVPSRFSGSGYGTDFTLTISSLQPEDFATYYCLQTNNLPLTFGQGTKVEIKRTVAAPSVFIFPPSDEQLKSGTASVVCLLNNFYPREAKVQWKVDNALQSGNSQESVTEQDSKDSTYSLSSTLTLSKADYEKHKVYACEVTHQGLSSPVTKSFNRGEC

SEQ ID NO: 90 - DNA, 642 bp, synthetic construct
  source 1..642: mol_type = other DNA
gatatccaaatgactcaaagtccaagtagtctctctgcttctgtcggcgacagagtgaccatcacctgtatcacctccaccgacatcgacgaggacatgaattggtatcagcagaaaccaggcaaggcccctaagctgctgatctacgaggacaactccctgcggcctggcgtgccctccagattcagcggatctggctacggcacagatttcaccctgacaatctccagcctgcaacctgaggattttgccacctactactgcctgcagaccaacaacctgcctctgaccttcggccagggcaccaaggtggaaatcaagcgtacggtggccgctcccagcgtgttcatctttcccccttctgacgagcagctgaagtctggcaccgcttccgtggtgtgcctgctgaacaatttctaccccagagaggccaaggtgcagtggaaggtggataacgctctgcagtccggcaatagccaggagtctgtgaccgagcaggactccaaggatagcacatattctctgtcttccaccctgacactgtctaaggccgactacgagaagcacaaggtgtatgcttgcgaggtgacccatcagggcctgagctctcctgtgacaaagtcctttaatcgcggcgagtgt

SEQ ID NO: 91 - protein, 214 aa, synthetic construct
DIQMTQSPSSLSASVGDRVTITCITSTDIDEDMNWYQQKPGKAPKLLISEDNSLRPGVPSRFSSSGYGTDFTLTISSLQPEDFATYYCLQTNNLPLTFGQGTKVEIKRTVAAPSVFIFPPSDEQLKSGTASVVCLLNNFYPREAKVQWKVDNALQSGNSQESVTEQDSKDSTYSLSSTLTLSKADYEKHKVYACEVTHQGLSSPVTKSFNRGEC

SEQ ID NO: 92 - DNA, 642 bp, synthetic construct
  source 1..642: mol_type = other DNA
gatatccaaatgactcaaagtccaagtagtctctctgcctccgtgggcgacagagtgaccatcacctgtatcacctccaccgacatcgacgaggacatgaattggtaccagcagaaacctggcaaggcccctaagctgctgatctccgaggacaactccctgagaccaggagtccccagccggttctccagctctggctacggcacagatttcaccctgacaatctcttctctgcaacctgaggattttgctacctactactgcctgcagaccaacaacctgcctctgaccttcggccagggcaccaaggtggaaatcaagcgtacggtggccgctcccagcgtgttcatctttcccccttctgacgagcagctgaagtctggcaccgcttccgtggtgtgcctgctgaacaatttctaccccagagaggccaaggtgcagtggaaggtggataacgctctgcagtccggcaatagccaggagtctgtgaccgagcaggactccaaggatagcacatattctctgtcttccaccctgacactgtctaaggccgactacgagaagcacaaggtgtatgcttgcgaggtgacccatcagggcctgagctctcctgtgacaaagtcctttaatcgcggcgagtgt

SEQ ID NO: 93 - protein, 611 aa, synthetic construct
QETELSVSAELVPTSSWNISSELNKDSYLTLDEPMNNITTSLGQTAELHCKVSGNPPPTIRWFKNDAPVVQEPRRLSFRSTIYGSRLRIRNLDTTDTGYFQCVATNGKEVVSSTGVLFVKFGPPPTASPGYSDEYEEDGFCQPYRGIACARFIGNRTVYMESLHMQGEIENQITAAFTMIGTSSHLSDKCSQFAIPSLCHYAFPYCDETSSVPKPRDLCRDECEILENVLCQTEYIFARSNPMILMRLKLPNCEDLPQPESPEAANCIRIGIPMADPINKNHKCYNSTGVDYRGTVSVTKSGRQCQPWNSQYPHTHTFTALRFPELNGGHSYCRNPGNQKEAPWCFTLDENFKSDLCDIPACDSKDSKEKNKMEIEGRMDPKSSDKTHTCPPCPAPELLGGPSVFLFPPKPKDTLMISRTPEVTCVVVDVSHEDPEVKFNWYVDGVEVHNAKTKPREEQYNSTYRVVSVLTVLHQDWLNGKEYKCKVSNKALPAPIEKTISKAKGQPREPQVYTLPPSRDELTKNQVSLTCLVKGFYPSDIAVEWESNGQPENNYKTTPPVLDSDGSFFLYSKLTVDKSRWQQGNVFSCSVMHEALHNHYTQKSLSLSPGK

SEQ ID NO: 94 - protein, 392 aa, synthetic construct
QETELSVSAELVPTSSWNISSELNKDSYLTLDEPMNNITTSLGQTAELHCKVSGNPPPTIRWFKNDAPVVQEPRRLSFRSTIYGSRLRIRNLDTTDTGYFQCVATNGKEVVSSTGVLFVKFGPPPTASPGYSDEYEEDGFCQPYRGIACARFIGNRTVYMESLHMQGEIENQITAAFTMIGTSSHLSDKCSQFAIPSLCHYAFPYCDETSSVPKPRDLCRDECEILENVLCQTEYIFARSNPMILMRLKLPNCEDLPQPESPEAANCIRIGIPMADPINKNHKCYNSTGVDYRGTVSVTKSGRQCQPWNSQYPHTHTFTALRFPELNGGHSYCRNPGNQKEAPWCFTLDENFKSDLCDIPACDSKDSKEKNKMEGGGSGGGSHHHHHHHHHH

SEQ ID NO: 95 - protein, 937 aa, synthetic construct
MHRPRRRGTRPPLLALLAALLLAARGAAAQETELSVSAELVPTSSWNISSELNKDSYLTLDEPMNNITTSLGQTAELHCKVSGNPPPTIRWFKNDAPVVQEPRRLSFRSTIYGSRLRIRNLDTTDTGYFQCVATNGKEVVSSTGVLFVKFGPPPTASPGYSDEYEEDGFCQPYRGIACARFIGNRTVYMESLHMQGEIENQITAAFTMIGTSSHLSDKCSQFAIPSLCHYAFPYCDETSSVPKPRDLCRDECEILENVLCQTEYIFARSNPMILMRLKLPNCEDLPQPESPEAANCIRIGIPMADPINKNHKCYNSTGVDYRGTVSVTKSGRQCQPWNSQYPHTHTFTALRFPELNGGHSYCRNPGNQKEAPWCFTLDENFKSDLCDIPACDSKDSKEKNKMEILYILVPSVAIPLAIALLFFFICVCRNNQKSSSAPVQRQPKHVRGQNVEMSMLNAYKPKSKAKELPLSAVRFMEELGECAFGKIYKGHLYLPGMDHAQLVAIKTLKDYNNPQQWTEFQQEASLMAELHHPNIVCLLGAVTQEQPVCMLFEYINQGDLHEFLIMRSPHSDVGCSSDEDGTVKSSLDHGDFLHIAIQIAAGMEYLSSHFFVHKDLAARNILIGEQLHVKISDLGLSREIYSADYYRVQSKSLLPIRWMPPEAIMYGKFSSDSDIWSFGVVLWEIFSFGLQPYYGFSNQEVIEMVRKRQLLPCSEDCPPRMYSLMTECWNEIPSRRPRFKDIHVRLRSWEGLSSHTSSTTPSGGNATTQTTSLSASPVSNLSNPRYPNYMFPSQGITPQGQIAGFIGPPIPQNQRFIPINGYPIPPGYAAFPAAHYQPTGPPRVIQHCPPPKSRSPSSASGSTSTGHVTSLPSSGSNQEANIPLLPHMSIPNHPGGMGITVFGNKSQKPYKIDSKQASLLGDANIHGHTESMISAEL